European Patent Application EP 4 782 532 A1, published July 29, 2026. Title: Butanol-producing Hydrogenophilus bacterium transformant. Applicant: 株式会社ＣＯ２資源化研究所. The sequence listing filed with the application follows.

SEQUENCE LISTING (62 sequences)

SEQ ID NO: 1 - DNA, 2619 bp, Thermoanaerobacter mathranii
  source 1..2619: mol_type = genomic DNA
atgcctactttattacaagaaaaaaaggaaacaaaagaaaaaacagaagtaaaagaaacaacagatgttaaaaaacaaatagacctattagtagaaagggcaaaaagagcccaagaaaaattcatgtcatacactcaagagcaaattgatgaaatagtcaaagttatggcactagcgggcatagaaaagcatgtagaactggcaaaattagctcatgaagaaacgaaaatgggggtttatgaagacaaaataacgaaaaatctctttgcagtagaatatgtgtacaattatataaaagacaaaaagactgtcggcatccttagtgaaaacttagaagaaaatcatatggaagtggcagagcctgtaggaattatagcaggggttacccccgtgacaaaccctacctctacaacaatgtttaaatgcttaatagctatcaaaacaagaaatccaataatttttagtttccatcccaaagcattaaaatgtagtatagaagcagcaaagaccatgtacgaggcagcattaaaggcgggtgctcccgaaggatgcataggttggattgaaacaccttcaattgaagcaacgcaacttctcatgacacaccccggcgtctcccttatcctcgcaacaggcggtgcgggaatggtaaaagctgcttacagctcaggaaaacccgcccttggcgtaggtcctggcaatgtcccctgctacattgaaaaaactgcaaatattaaaagagcggtctcagacctaatacttagcaaaacttttgacaatggcacagtatgcgcatcagaacaagctgtgataatagatgaagaaatagccaatgaagtaaaaaaattaatgagagaatatggttgctatttcttaaataaagaagaaactaaaaagttagaagaattcgctatagacaaaaacaccggtttaatgaatccagcagttgtgggtcagcctgcagtgaaaattgctcaaatggctggatttaaagttcctgaaaataccaaaatacttgtagctgaatatccagctgtaggtcctaaatatcctctatccagagaaaaactaagcccaatacttgctttatacacagtcaaagattacaaagaaggtataaaaagatgcgaagaaatgatacaattcggcggacttggtcactctgcggtaatacattctgaaaaccaacaaattattaatgaatttgcaaatagagtacaagcaagtagaatccttgtaaacgcccctgcttcacaaggcgctattggagacatttataacacggctactccatctttgactttgggttgcggtacaatgggtggaaattcaacaacagataatgtaagtgtttataaccttataaacataaaacgagtttttataagaaaagagagaatgaaatggttcagagttccaccacaaatctattttgaaagagggtcaatacagtatctatcacaagtaaaaggcaaaaaagcttttattgtaacagaccctgcaatggttaaattaggttttgtagataaagtgacatatcaattagataaagcaaatattaaatatgaaattttctctgaagtagaaccagacccatcagttgacactgtagaaaaagggataaaaataatgaaggagttcgagcctgacttactaatagctgtaggtggtggttctgcaatagacgcagcaaagggaatgtggcttttttatgagtaccctgacacaaaatttgaagacttaaggttaaagttcatggacataagaaaaagaacttatagatttcctgaactcggcaaaaaagctttatttatcgcaataccaaccaccagcggtacaggttctgaagtcacagcctttgcagttataacagacaaaaagaaaaatataaagtaccctcttacagattacgaattgacaccagatattgctataatagaccctgactttgtcatgacaattccaccctctgtaactgcagatacaggtatggatgctttaactcatgccattgaagcttatgtatccgtgatggcatcagactatacagacgccctcgcagaaaaagccataaaactgatatttgaatatctccctaaagcatataaaaacggacaagacaaagtcgcccgcgaaaagatgcacaatgcttcttgcatagcaggaatggcattcacaaatgcatttttaggaataaaccacagtatggcccacatacttggcgctaaattccaccttccccatggaagggcaaatgcgatacttctgccctatgtcatagaatacaatgctgagttacctaaaaaatttgcctcattcccacaatatgaatatcccaaagcagccgagaaatacgcagaaattgcaaaattcttaggacttcctgcatcaaccactgatgaaggagtaaaaagtctcattgaagcaataaaaaatctcatgaaagagttaaatcttcctcttacacttaaagatgcgggaataaacaaagaagaatttgaaaaacaaataatggaaatggctgatatagccttcaacgaccagtgcaccggttcaaatccaagaatgccattggtatcagaaattgcagaaatatatagaaaagcctatggagaataa

SEQ ID NO: 2 - protein, 872 aa, Thermoanaerobacter mathranii
MPTLLQEKKETKEKTEVKETTDVKKQIDLLVERAKRAQEKFMSYTQEQIDEIVKVMALAGIEKHVELAKLAHEETKMGVYEDKITKNLFAVEYVYNYIKDKKTVGILSENLEENHMEVAEPVGIIAGVTPVTNPTSTTMFKCLIAIKTRNPIIFSFHPKALKCSIEAAKTMYEAALKAGAPEGCIGWIETPSIEATQLLMTHPGVSLILATGGAGMVKAAYSSGKPALGVGPGNVPCYIEKTANIKRAVSDLILSKTFDNGTVCASEQAVIIDEEIANEVKKLMREYGCYFLNKEETKKLEEFAIDKNTGLMNPAVVGQPAVKIAQMAGFKVPENTKILVAEYPAVGPKYPLSREKLSPILALYTVKDYKEGIKRCEEMIQFGGLGHSAVIHSENQQIINEFANRVQASRILVNAPASQGAIGDIYNTATPSLTLGCGTMGGNSTTDNVSVYNLINIKRVFIRKERMKWFRVPPQIYFERGSIQYLSQVKGKKAFIVTDPAMVKLGFVDKVTYQLDKANIKYEIFSEVEPDPSVDTVEKGIKIMKEFEPDLLIAVGGGSAIDAAKGMWLFYEYPDTKFEDLRLKFMDIRKRTYRFPELGKKALFIAIPTTSGTGSEVTAFAVITDKKKNIKYPLTDYELTPDIAIIDPDFVMTIPPSVTADTGMDALTHAIEAYVSVMASDYTDALAEKAIKLIFEYLPKAYKNGQDKVAREKMHNASCIAGMAFTNAFLGINHSMAHILGAKFHLPHGRANAILLPYVIEYNAELPKKFASFPQYEYPKAAEKYAEIAKFLGLPASTTDEGVKSLIEAIKNLMKELNLPLTLKDAGINKEEFEKQIMEMADIAFNDQCTGSNPRMPLVSEIAEIYRKAYGE

SEQ ID NO: 3 - DNA, 2613 bp, Fonticella tunisiensis
  source 1..2613: mol_type = genomic DNA
atgaaagtaacaaatgcagaagaactaagattaaagcttgaggaggttagaaaagcccaaaaaatattcgcctcctacacccaggaacaggtagatgaaatatttagacaggctgctatggctgctaacaatgcaagaattaagcttgcaaagatggctgttgaagaaacaggaatgggaattgtagaagacaaagttattaaaaaccactttgcctcagaatatatatacaataaatataaggatgaaaagacctgcggagttattgacagagatgaatccttcggcataatgagggttgcagaacctataggagttatcgctgcaatagtaccaactaccaacccgacatccactgcaatatttaaagcattaatcgctttaaaaacaagaaacggtgtgattttctcaccccatccaagggctaaaaaatcaactatagcagcagctaaaatcgtacttgatgctgcagttaaggccggtgcccctgagggaataataggatggattgatgaaccaacggttgaactttcacagatcgttatgaaggaagctgatatgatacttgccacaggcggccccggaatggtaagagctgcttattcctcaggaaaacccgcaataggagtaggtgctggaaatacgcctgcaataatagatgaaacagcacatattaaaatggcagtaagctccatacttctttcaaagacatttgacaacggagttatatgtgcttcagaacagtcagtaattgtaatggaacaaatatatgacgaagttaagcgtgagtttgaggaaagaggagcatacttcctaaagggagaggaaatcgacaaggttagaaagataatacttgttaatggttcaataaatgcaaatatagttggacagcctgcccacaaaatagctgaaatggctggagttaaagttcctgaaacagcaaaggtattaatcggagaagttgaatccgttgaactcgatgaaccattctcacacgaaaaactttcacctgtgctcgctatgtataaggctaaaaccttcgatgaggcacttcagaaagctgcaaggcttgtggaacttggcggatttgggcatacatcagttctatataccgaccaggtaaaatcaagggatagaattgaaaaatttggtgcgactatgaagacaggaagaacaataatcaatatgccttcgtcccaaggtgcaataggagatatctataacttcaggcttgctccttcgctaacactcggatgtggtacatggggtggaaactctgtatctgaaaacgttggagttaagcatcttttaaacatcaagagtgttgctgaaaggagagaaaatatgctttggttcagagttcctgaaaagatatacttcaaatacggctgcctgcctgtagcattaaaggaattaaaggatatgggcaagaagagggcattcatcgttactgacaaagttctgtataatttaggatttatcgatacagttacaaagacccttgatgaaataggaattgaatatagcgtgttctttgacgttgaaccagacccaacacttgcaactgcaagaaagggtgcagcacaaatgaaaagcctcaatccggatgtaataattgcagttggtggaggctcacctatggatgctgcaaagattatgtgggtactttatgagcatccggaagtaaggtttgaagaccttgcaatgagatttatggatattagaaagagagtttaccagttcccaaagatgggcgaaaaggctatgatggtttcaatcccaacttcttccggaacaggttcagaggttactccatttgctgttataaccgatgaaaagacgggaattaaatatcctcttgcagactatgagttaactcctgatatggcaatagtagatgcagaacttatgctcaatatgccaaagggacttacagcagcatctggtatagacgccctaactcatgcaatagaagcctatgtttcggtacttgcatcagagtatactaacggacttgcccttgaagcgataagacttatattcaaatatctaccacaggcatataatgatggtccaaacaacatcaaagcaagggaaaagatggcccacgctgcaactatggctggtatggcctttgcaaatgcattcctcggcgtatgccactcaatggcccacaagcttggagcaatgcatcatgtaccacacggagttgccaacggccttctaattaacgaagtaataagatttaatgcagttgataacccaagaaagcaaactgcattcccacagtataaatatccaaacgccaagttcagatatgcaaggattgctgactacctgaaccttggcggaaataccgaagatgaaaagattgaactccttataaaggcaatcgacgacttaaagaaccaggttaacatgccaaaaacgataagtgaagctggtgtttcaagagagaaattctacgcaacccttgatgaaatgtgcgaacaggccttcgacgaccagtgcacaggtgccaacccaagatatccgttaataagcgaaatcaagcagatgtatataaacgctttcgaaggaatttcaaaggaaactgaagaaaataataaataa

SEQ ID NO: 4 - protein, 870 aa, Fonticella tunisiensis
MKVTNAEELRLKLEEVRKAQKIFASYTQEQVDEIFRQAAMAANNARIKLAKMAVEETGMGIVEDKVIKNHFASEYIYNKYKDEKTCGVIDRDESFGIMRVAEPIGVIAAIVPTTNPTSTAIFKALIALKTRNGVIFSPHPRAKKSTIAAAKIVLDAAVKAGAPEGIIGWIDEPTVELSQIVMKEADMILATGGPGMVRAAYSSGKPAIGVGAGNTPAIIDETAHIKMAVSSILLSKTFDNGVICASEQSVIVMEQIYDEVKREFEERGAYFLKGEEIDKVRKIILVNGSINANIVGQPAHKIAEMAGVKVPETAKVLIGEVESVELDEPFSHEKLSPVLAMYKAKTFDEALQKAARLVELGGFGHTSVLYTDQVKSRDRIEKFGATMKTGRTIINMPSSQGAIGDIYNFRLAPSLTLGCGTWGGNSVSENVGVKHLLNIKSVAERRENMLWFRVPEKIYFKYGCLPVALKELKDMGKKRAFIVTDKVLYNLGFIDTVTKTLDEIGIEYSVFFDVEPDPTLATARKGAAQMKSLNPDVIIAVGGGSPMDAAKIMWVLYEHPEVRFEDLAMRFMDIRKRVYQFPKMGEKAMMVSIPTSSGTGSEVTPFAVITDEKTGIKYPLADYELTPDMAIVDAELMLNMPKGLTAASGIDALTHAIEAYVSVLASEYTNGLALEAIRLIFKYLPQAYNDGPNNIKAREKMAHAATMAGMAFANAFLGVCHSMAHKLGAMHHVPHGVANGLLINEVIRFNAVDNPRKQTAFPQYKYPNAKFRYARIADYLNLGGNTEDEKIELLIKAIDDLKNQVNMPKTISEAGVSREKFYATLDEMCEQAFDDQCTGANPRYPLISEIKQMYINAFEGISKETEENNK

SEQ ID NO: 5 - DNA, 2718 bp, Thermoclostridium caenicola
  source 1..2718: mol_type = genomic DNA
atggaaaacaaagaaagaaagattgtagacagtgtggacgcgttaaagaaagtcattgcccgggtaagggaagcgcaaaggaaattttcaacctattcccaggaacaggtggatgaaatttttaaggctgctgccactgccgcaaaccaggcaagaattccgctggcgaaaatggcggtggaagaaaccggtatgggcgttgtggaagataaagttataaaaaaccactatgccgccgaatatgtttacaatacgtataagaacgtaagaacctgcggggttttggaagaagataaggcatacggtatcaaaaaaattgccgagcctgtcggtgtgattgccgctgttattcctaccactaaccctacttccacggcaatttttaaaaccctgatcgcgctgaaaacacgcaatgccgttattatcagcccacatccgagagctaaaaaatgcaccatcgctgcggcaaaaatcgtattggatgctgccgttgccgcgggggctccggaagggattattgactggattgatgtgccgaacattgagttgaccaatctgcttatgaaagaagcagacattatccttgccacaggtggtcccggtatggtgaaggcggcttattcctccgggaaaccggctatcggtgtcgggcctggcaatactccggccgttattgatgaaagcgccgacgttgtccttgccgtgaactccattattcattccaaaacgtttgataatggtatgatttgcgcatcagaacaatcggtaattgttcacaagaatgtttatgacgctgtaaaagctgaatttgcggcccgtggatgctatttccttaaagaagatgaaattgaaaaggtacgcaagacgatttttgtcaacggcgcgttaaatgcccagattgttggtcagccggcatacaaaattgccgaacttgccggtgtgaaagtgcctgtaggcacaaaaatcctcatcggagaagttgacagcacagacccgtcggaagaatttgcccatgaaaagctgtcacctgtccttgcgatgtataaagctgaggatattcatgacgcttttgagaaagccgaacgtttggttgccaacggaggttacggtcataccgcagcaatttatttggatgtaaccaccgaacaggctaaaattgacgaattcgcttcgcgtttgaagacctgccgtatacttgtgaatactccgtcttctcagggagctatcggcgacatttacaactttaagcttgcgccgtcgttaactcttggctgtggttcctggggcggaaattcggtttccgaaaatgttggggtaaaacacctgcttaatatcaaaacggttgttgaaagaagggaaaatatgctgtggttccgcgctcccgaaaaaatatacatcaaaaagggatgtttgccggtagcccttaatgagttgaaatacgtcatgggtaagaaacgcgcttttatagttaccgacagcttcctctatcacaatggttacacaaagcccattaccgacagacttgacgaactgggcattgaacatacaacgttttttgatgttttacccgatccgacgctttcctgcgcaaaagcgggagctgagcagatgagagccttccagcccgataccattattgccttcggtggcggatctgcgatggacgccgcgaaaatcatgtgggtaatgtatgagcatcccgaagttgatttcatggacatggctatgcgttttatggatatcaggaaaagggtttatacatttccgaaaatgggagaaaaggcgtattttgttgcaataccgacttctgcgggtaccggatccgaagtaactccttttgcggttatcaccgacgaaaagagtggagtaaaatatcccctcgcagactacgagttgctccccgacatggcaattatagatgtggattttcacatgagtgctcccaagggccttaccgccgcagcaggtatagatgccctcacccatgcgcttgaggcgtacgtttctcttatggccactgattttaccgacggactggcgaaacaggctctgcagatgatttttaaatacctgccccgcgcctatgataacggtcagaccgatgtggaagcacgtgaaaaaatggctaatgccgccaccattgcaggtatggcgtttgcaaatgctttccttggtgtttgccattccatggcacataagctgggcgctttttatcatttgcctcatggtattgccaacgcgcttatgatagaagaagtaatccgtttcaacgcttcggaagcaccggccaaaatgggaactttcccgcaatacggatacccgcacgctttaagacgttatgccgaaattgctgaggcgcttaatctcggcggcgaaaacgatcatgaaaagctggaaaatctcattaaagccattaatgatctgaaggcaagggtggggatcaagtcatcaatcaaagagtatggcataaatgagaaggaattcctggaacgcctcgacgagatggttgaacaggcattcgacgaccagtgcaccggtaccaatccgcgatatccgctgatgagcgaaataaggcaaatgtatctgaatgcttattacggcaaaaaacattttgtcgatgaagaaaagccaaatgaagcggatatcgccgggacagaggatgaaaacaaagttaaaaaggcgtatctgagagccagagtcggagcgaagagagcatga

SEQ ID NO: 6 - protein, 905 aa, Thermoclostridium caenicola
MENKERKIVDSVDALKKVIARVREAQRKFSTYSQEQVDEIFKAAATAANQARIPLAKMAVEETGMGVVEDKVIKNHYAAEYVYNTYKNVRTCGVLEEDKAYGIKKIAEPVGVIAAVIPTTNPTSTAIFKTLIALKTRNAVIISPHPRAKKCTIAAAKIVLDAAVAAGAPEGIIDWIDVPNIELTNLLMKEADIILATGGPGMVKAAYSSGKPAIGVGPGNTPAVIDESADVVLAVNSIIHSKTFDNGMICASEQSVIVHKNVYDAVKAEFAARGCYFLKEDEIEKVRKTIFVNGALNAQIVGQPAYKIAELAGVKVPVGTKILIGEVDSTDPSEEFAHEKLSPVLAMYKAEDIHDAFEKAERLVANGGYGHTAAIYLDVTTEQAKIDEFASRLKTCRILVNTPSSQGAIGDIYNFKLAPSLTLGCGSWGGNSVSENVGVKHLLNIKTVVERRENMLWFRAPEKIYIKKGCLPVALNELKYVMGKKRAFIVTDSFLYHNGYTKPITDRLDELGIEHTTFFDVLPDPTLSCAKAGAEQMRAFQPDTIIAFGGGSAMDAAKIMWVMYEHPEVDFMDMAMRFMDIRKRVYTFPKMGEKAYFVAIPTSAGTGSEVTPFAVITDEKSGVKYPLADYELLPDMAIIDVDFHMSAPKGLTAAAGIDALTHALEAYVSLMATDFTDGLAKQALQMIFKYLPRAYDNGQTDVEAREKMANAATIAGMAFANAFLGVCHSMAHKLGAFYHLPHGIANALMIEEVIRFNASEAPAKMGTFPQYGYPHALRRYAEIAEALNLGGENDHEKLENLIKAINDLKARVGIKSSIKEYGINEKEFLERLDEMVEQAFDDQCTGTNPRYPLMSEIRQMYLNAYYGKKHFVDEEKPNEADIAGTEDENKVKKAYLRARVGAKRA

SEQ ID NO: 7 - DNA, 2619 bp, Thermoanaerobacter ethanolicus
  source 1..2619: mol_type = genomic DNA
atgcctaacttattacaagaaagaagagaagtaaaagaaaaaacagaagtgaaagaaacgctggatgttaaaagacaaatagaccaattagtagaaaaagcacaaagagcacaagaaaaattcatgtcttatacccaagaacaaatagataaaatagttaaagctatggctttggctggtattgaaaatcatgtgagattggcaaaattagcccatgaagaaacaaaaatgggtgtttatgaagacaaaataacgaaaaatctttttgcagtagaatatgtgtacaattatataaaagacaaaaagactgtcggcgtccttagtgaaaacttagaagaaaattatatggaagtggcagaacctgtaggagttatagccggcgtaacacccgttacaaaccctacttctacaacaatgttcaaaagcttaatcgctattaaaacaagaaatccaataatttttagctttcacccaaaagcattaaaatgtagtatagaaacagcaaagaccatgtacgaggcagcattaaaagctggtgcaccagaaggatgcataggttggattgaaacgccttcaattgaagcaacgcaacttctcatgacacatcccggcgtctcccttatcctcgcaacaggcggcgctggaatggtaaaagccgcttacagctcaggaaaacccgcccttggcgtaggtcctggcaatgtcccctgctacattgaaaaaactgcaaatattaaaagagcagtctcagacctaatacttagcaaaacttttgacaatggcacagtatgcgcatcagaacaagctgtgataatagacgaagaaatagcagatgaagtgaaaaaaaatatgaaagaatatggttgctattttctcaataaagaagagactaaaatgctagaagaattcgctatagacaaaaacaccggtttaatgaatccagcagttgtaggtcaaccggcaacaaaaattgctgaaatggctggatttaaagtacctgaaaacacaaaaatacttgtagctgaatatcctgctgtaggaccagaatatcctctctccagagaaaagctaagtccaatacttgctttatacacagtcaaagattacaacgaaggcataaaaagatgtgaagaaatgacagaattcggcggacttggtcactctgcagtaatacattctgaaaaccaacaaattattaatgaatttgcaaaaagagtacgagcaggaagaattcttgtaaacgcccctgcttctcaaggagctattggagatatttataacacggctatcccatctttgactttgggttgcggtacaatgggtagaaattcaacaacagataatgtaagtgtttataaccttataaacataaaacgagtttttataagaaaagagagaatgaaatggttcagagttccaccacaaatttattttgaaagagggtcattacaatatctgtcacaagtaaaaggcaaaaaagcctttattgtaacagaccctgtgatggttaaattaggttttgtagataaagtaacgtatcaattagataaggcaaatattaaatatgaaatattctctgaagttgaaccagatccttcagttgacactgtagaaaaaggggtaaaaataatgagagggtttgagcctgacttactaatagctgtaggtggtggttctgcaatagatgcagcgaagggaatgtggcttttctacgaataccctgatacaaaattcgaagacttaaggttaaaatttatggacataagaaaaagaacttatagatttcctgaactggggaaaaaagctttatttatcgcaataccaaccaccagcggtacaggttctgaagttactgcctttgcagttataacagacaaaaagaaaaatataaagtaccctctcacagattacgaattaacaccagatatcgctataatagaccctgacctcacaatgacaataccaccctctgtcacagcagacactggtatggacgctttaacccatgctattgaagcctatgtatctgtaatggcatcagactatacagacgctctcgcagaaaaagctataaaattgatatttgaatatctacctaaagcatacaaaaacgggcaagataaagtcgcccgcgaaaagatgcacaatgcttcatgcatagctggaatggccttcacaaatgcatttttaggaataaaccatagtatggctcatatacttggtgctaaattccatcttccacacggaagagcaaatgcaatacttctgccctatgtcatagaatacaatgctgagttacctaaaaaatttgcttcattcccacaatatgaatatcccaaagcagccgagaaatatgcagaaattgcaaaattcttgggacttcctgcatcaaccattgaagaaggagtaaaaagcctcattgaagcaataaaaaatcttatgaaagagcttaatcttcctttgacacttaaagaagcaggcataaataaagaagaattcgaaaaacaaataatggaaatgtctgatatagcctttaatgaccagtgcaccggttcaaacccaagaatgccattggtatccgaaattgcagaaatatatagaaaagcctatggagaataa

SEQ ID NO: 8 - protein, 872 aa, Thermoanaerobacter ethanolicus
MPNLLQERREVKEKTEVKETLDVKRQIDQLVEKAQRAQEKFMSYTQEQIDKIVKAMALAGIENHVRLAKLAHEETKMGVYEDKITKNLFAVEYVYNYIKDKKTVGVLSENLEENYMEVAEPVGVIAGVTPVTNPTSTTMFKSLIAIKTRNPIIFSFHPKALKCSIETAKTMYEAALKAGAPEGCIGWIETPSIEATQLLMTHPGVSLILATGGAGMVKAAYSSGKPALGVGPGNVPCYIEKTANIKRAVSDLILSKTFDNGTVCASEQAVIIDEEIADEVKKNMKEYGCYFLNKEETKMLEEFAIDKNTGLMNPAVVGQPATKIAEMAGFKVPENTKILVAEYPAVGPEYPLSREKLSPILALYTVKDYNEGIKRCEEMTEFGGLGHSAVIHSENQQIINEFAKRVRAGRILVNAPASQGAIGDIYNTAIPSLTLGCGTMGRNSTTDNVSVYNLINIKRVFIRKERMKWFRVPPQIYFERGSLQYLSQVKGKKAFIVTDPVMVKLGFVDKVTYQLDKANIKYEIFSEVEPDPSVDTVEKGVKIMRGFEPDLLIAVGGGSAIDAAKGMWLFYEYPDTKFEDLRLKFMDIRKRTYRFPELGKKALFIAIPTTSGTGSEVTAFAVITDKKKNIKYPLTDYELTPDIAIIDPDLTMTIPPSVTADTGMDALTHAIEAYVSVMASDYTDALAEKAIKLIFEYLPKAYKNGQDKVAREKMHNASCIAGMAFTNAFLGINHSMAHILGAKFHLPHGRANAILLPYVIEYNAELPKKFASFPQYEYPKAAEKYAEIAKFLGLPASTIEEGVKSLIEAIKNLMKELNLPLTLKEAGINKEEFEKQIMEMSDIAFNDQCTGSNPRMPLVSEIAEIYRKAYGE

SEQ ID NO: 9 - DNA, 2613 bp, Bacillus coagulans
  source 1..2613: mol_type = genomic DNA
atggcaatcgatgaaaaagttgttggcaaatctgcgcaaatcacggaaatggtcgattccctcgtcgcaaaagggcaaaaagcactgcgtgaatttatggaactggatcaggcacaagtggacaatatcgtaaaacaaatggcacttgccgggttggaacagcatatggtgctcgccaaaatggccgtggaagaaacagggcgcggcgtatatgaagacaaaatgacaaaaaacttgtttgcaacagaatacatctatcacaacattaaatataacaaaacagtcggcatcattgacgaaaacaataatgaagggattgttaaatttgcggaaccggtcggcgtgattgccggggtcactcctgtaacaaacccgacatcaaccacgatgtttaaagcattaattgccattaaaacacgcaacccaattattttcgcgttccatccgtccgcacaaaaatgcagcagccatgccgcaaaagtgatgcttgacgctgctgtgaaagccggcgccccggaaaactgcatccaatggatcgaaaaaccggccattgaagcgacacagcaattgatgaaccattcgggtatttcactgattcttgcaacgggcggttccggcatggtaaagtccgcatattcgagcgggaaacctgcgcttggcgtcgggccgggaaacgtcccttgctatattgaaaaatctgctgatatcaaacgcgccgtcaatgatttgattttgtccaaaacgtttgacaacggcatgatctgtgcgtcggaacaggctgtcatcatcgacaaagaaatttatgacaatgtgaaaaacgaattgattgcaaatcaatgctacttcctgaatgaagcggagaagaaaaaggttgagaaaaccgtcatcaatgaaaagacgcaatccgtcaacagcgccattgtcggcaaaccggcctatgaaattgcgaaaatggcaggcgtaaatgttccggaagataccaaaattttaatcgccgaacttacaggtgtcggcccggactacccgctttccagagaaaaattaagcccggttttggcctgttacaaagccaacagcacaaaacaaggtttcgaatttgcagaagccatgctcgaattcggcggacttggtcactcggctgtgatccattcgacaaacgatgaagtcattgaacaatacggcttaaaaatgaaagccggccggatcattgtcaactccccgtcttcgcaaggggcaatcggcgacatttacaatgcctacatgccttctttgacactcggctgcggcacgtttggcggcaactcggtgtccacaaacgtcggtgtcatcaatctttacaatgtaaaaacaatggcgaaacggagagtcaatatgcaatggtttaaaattccaccgcgcgtgtattttgaaaagaactcggtccaatacctggaaaaaatgccggatatctcaagtgcctttattgtcaccgatccggatatggtcaggcttggattcgttgagaaagtactgtattacttgcggaaacgcccggactatgtgcactgtgaaattttctcagaagtcgaaccggatccgtctattgaaacggttcggaaaggtgccgcagctatggcaagcttccagccggatgtcattatcgcgcttggcggcgggtcggcgatggatgctgcaaaaggcatgtggctgttctatgagcatccggaagttgatttcaacgaattgaagcaaaaatttatggacatccggaaacgggttgccaaattcccgaaactgggtgaaaaagcgcagctggtctgcattccgaccacatcgggcaccggttctgaagtgacttctttcgccgtcatttcggataaaaagaacaacacaaaatatccgctcgcagactatgaactgacaccggatgttgcgatcattgacccgcagtttgttatgaccgttccgaaatccgtaacagccgataccgggatggacgttttgacccatgcgattgaagcctatgtatccaacatggccaacgactatacggacggcctggcaattaaggccatccagcttgttcacgaatacttgccgaaagcatacgcaaatggcaatgatgcactggcacgcgaaaaaatgcacaatgcatcgactttggcagggatggcgttctcgaatgcattccttggcatcaaccattcacttgcccataaaatcggcgctgaattccatattccgcacggccgggctaacgcgattctgttgccgcatgtcatccgctataacgcgcaaaagccgaaaaaatttgcggcattcccgaaatacgaacattttattgcggatcaacgctacgcggaaatcgcgcgcgtacttggtcttccggcaagcacgacagaagaaggtgtcgaaagcctttgccaggaaatcatccggatgtgcaaactgttcaatattccgcttagcctaaaagcagccggcgtgaaccgggcggactttgaaaaacgggttgccattattgcagaccgcgcatttgaagaccaatgcacacctgcaaaccctaaattgccgcttgtcagcgaattggaagacattttacgcaaagcttttgaaggcgttgaagcaaaataa

SEQ ID NO: 10 - protein, 870 aa, Bacillus coagulans
MAIDEKVVGKSAQITEMVDSLVAKGQKALREFMELDQAQVDNIVKQMALAGLEQHMVLAKMAVEETGRGVYEDKMTKNLFATEYIYHNIKYNKTVGIIDENNNEGIVKFAEPVGVIAGVTPVTNPTSTTMFKALIAIKTRNPIIFAFHPSAQKCSSHAAKVMLDAAVKAGAPENCIQWIEKPAIEATQQLMNHSGISLILATGGSGMVKSAYSSGKPALGVGPGNVPCYIEKSADIKRAVNDLILSKTFDNGMICASEQAVIIDKEIYDNVKNELIANQCYFLNEAEKKKVEKTVINEKTQSVNSAIVGKPAYEIAKMAGVNVPEDTKILIAELTGVGPDYPLSREKLSPVLACYKANSTKQGFEFAEAMLEFGGLGHSAVIHSTNDEVIEQYGLKMKAGRIIVNSPSSQGAIGDIYNAYMPSLTLGCGTFGGNSVSTNVGVINLYNVKTMAKRRVNMQWFKIPPRVYFEKNSVQYLEKMPDISSAFIVTDPDMVRLGFVEKVLYYLRKRPDYVHCEIFSEVEPDPSIETVRKGAAAMASFQPDVIIALGGGSAMDAAKGMWLFYEHPEVDFNELKQKFMDIRKRVAKFPKLGEKAQLVCIPTTSGTGSEVTSFAVISDKKNNTKYPLADYELTPDVAIIDPQFVMTVPKSVTADTGMDVLTHAIEAYVSNMANDYTDGLAIKAIQLVHEYLPKAYANGNDALAREKMHNASTLAGMAFSNAFLGINHSLAHKIGAEFHIPHGRANAILLPHVIRYNAQKPKKFAAFPKYEHFIADQRYAEIARVLGLPASTTEEGVESLCQEIIRMCKLFNIPLSLKAAGVNRADFEKRVAIIADRAFEDQCTPANPKLPLVSELEDILRKAFEGVEAK

SEQ ID NO: 11 - DNA, 924 bp, Thermus thermophilus
  source 1..924: mol_type = genomic DNA
atgtccgaaagggttaaggtagccatcctgggctccggcaacatcgggacggacctgatgtacaagctcctgaagaacccgggccacatggagcttgtggcggtggtggggatagaccccaagtccgagggcctggcccgggcgcgggccttagggttagaggcgagccacgaagggatcgcctacatcctggagaggccggagatcaagatcgtctttgacgccaccagcgccaaggcccacgtgcgccacgccaagctcctgagggaggcggggaagatcgccatagacctcacgccggcggcccggggcccttacgtggtgcccccggtgaacctgaaggaacacctggacaaggacaacgtgaacctcatcacctgcggggggcaggccaccatccccctggtctacgcggtgcaccgggtggcccccgtgctctacgcggagatggtctccacggtggcctcccgctccgcgggccccggcacccggcagaacatcgacgagttcaccttcaccaccgcccggggcctggaggccatcgggggggccaagaaggggaaggccatcatcatcctgaacccggcggaaccccccatcctcatgaccaacaccgtgcgctgcatccccgaggacgagggctttgaccgggaggccgtggtggcgagcgtccgggccatggagcgggaggtccaggcctacgtgcccggctaccgcctgaaggcggacccggtgtttgagaggcttcccaccccctggggggagcgcaccgtggtctccatgctcctggaggtggagggggcgggggactatttgcccaaatacgccggcaacctggacatcatgacggcttctgcccggagggtgggggaggtcttcgcccagcacctcctggggaagcccgtggaggaggtggtggcgtga

SEQ ID NO: 12 - protein, 307 aa, Thermus thermophilus
MSERVKVAILGSGNIGTDLMYKLLKNPGHMELVAVVGIDPKSEGLARARALGLEASHEGIAYILERPEIKIVFDATSAKAHVRHAKLLREAGKIAIDLTPAARGPYVVPPVNLKEHLDKDNVNLITCGGQATIPLVYAVHRVAPVLYAEMVSTVASRSAGPGTRQNIDEFTFTTARGLEAIGGAKKGKAIIILNPAEPPILMTNTVRCIPEDEGFDREAVVASVRAMEREVQAYVPGYRLKADPVFERLPTPWGERTVVSMLLEVEGAGDYLPKYAGNLDIMTASARRVGEVFAQHLLGKPVEEVVA

SEQ ID NO: 13 - DNA, 1023 bp, Bacillus coagulans
  source 1..1023: mol_type = genomic DNA
atgagagcagcagtcgtcagttctgataagcaaaaactggtagaggtcaaagatgtgcagttgcgtccacttgaatatggggaagctttggtggatatcgaatactgcggtgtctgccatacggatctgcatgtggcaaagggcgactttggcgatgtgccgggacgcattctcggccatgaaggagtcggcattgtcagggaagtcgcggatggtgtcacttctcttaaagtgggagatcgtgtaagcgttgcctggttttttgaaggctgcgggcattgtgagtactgtttaacgggaaatgaaacattttgccgtgatgtgaaaaatgcaggctacagtgtcgacggagcaatggcagagcagtgcatcgtcaaagcggattacgccgtaaaagtgccggaagggctggatccaaggcaggcgacgagcattacttgcgcaggtgtcaccacttataaagccattaaagtcgcagatgtgaagccgggcgaatggattgccatttatggagccggcggtcttggtaaccttgctgtccagtacgccaaacatgtatttaatgcgaaagtcattgcgatcgatatcaatgacgacaaactttcactggcaaaagaagtcggtgctgatctcacctttaattccaaaatgaaaggcgatccggctgaatggatccaaaaagaagttggcggcgcgcatgctgcagtggtaacggctgtttcaaaacaggcttttaaccaggctgtccactctgtacggccggtttcaaaagtcgttgctgtcgggctccctccggaaacaatggatcttgaaattgtgaagacggttcttgacggaatagaagtcgtcggctctttggtaggcacgagaaaagaccttgaggaagcctttatgttcggggcggaaggaaaagtcgtcccggttgtgcacacgcgcagactggaagaagtgggagatgtgtttaaagaaatggaagaaggcagaatacagggcaggatggtcctggatatgtcgttgaaataa

SEQ ID NO: 14 - protein, 340 aa, Bacillus coagulans
MRAAVVSSDKQKLVEVKDVQLRPLEYGEALVDIEYCGVCHTDLHVAKGDFGDVPGRILGHEGVGIVREVADGVTSLKVGDRVSVAWFFEGCGHCEYCLTGNETFCRDVKNAGYSVDGAMAEQCIVKADYAVKVPEGLDPRQATSITCAGVTTYKAIKVADVKPGEWIAIYGAGGLGNLAVQYAKHVFNAKVIAIDINDDKLSLAKEVGADLTFNSKMKGDPAEWIQKEVGGAHAAVVTAVSKQAFNQAVHSVRPVSKVVAVGLPPETMDLEIVKTVLDGIEVVGSLVGTRKDLEEAFMFGAEGKVVPVVHTRRLEEVGDVFKEMEEGRIQGRMVLDMSLK

SEQ ID NO: 15 - DNA, 1014 bp, Zymomonas mobilis subsp. mobilis
  source 1..1014: mol_type = genomic DNA
atgaaagcagccgtcataactaaagatcatacgatcgaagtgaaagacaccaaattacgccctctgaaatacggggaagcgcttttggaaatggaatattgcggggtatgtcataccgatctccacgtgaaaaacggggattttggcgatgaaaccggcagaattaccggccatgaaggcatcggtatcgtcaagcaggtcggggaaggggttacttctctgaaagtcggtgaccgtgccagtgttgcatggttcttcaaaggctgcggccattgcgaatattgtgtcagtggaaatgaaacgctttgccgcaacgttgaaaatgccggttatacggttgacggcgctatggcagaagaatgcatcgtcgttgccgattactcggtcaaagtgccagatggtcttgatcctgcggttgccagcagcatcacttgcgcgggtgtaaccacctataaagcagtcaaagtttctcagatacagccgggacaatggctggctatctatggcttgggcggtttaggcaatctagcccttcaatatgccaagaatgttttcaacgccaaagtgatcgcgatcgatgtcaatgatgaacagctcgcttttgccaaagagctgggcgcagatatggtcatcaatccgaaaaacgaagatgctgccaaaatcattcaggaaaaagtcggcggcgcacatgcgacggtggtgacagctgttgccaaatccgcctttaactcggctgttgaggctatccgcgcgggtggccgtgttgtcgccgttggtctgcctcctgaaaaaatggatttgagcattcctcgcttggtgcttgacggtatcgaagtcttaggttctttggtcggaacgcgggaagatttgaaagaagccttccagtttgcagccgaaggtaaggtcaaaccgaaagtcaccaagcgtaaagtcgaagaaatcaaccaaatctttgacgaaatggaacatggtaaattcacaggccgtatggttgttgattttacccatcactag

SEQ ID NO: 16 - protein, 337 aa, Zymomonas mobilis subsp. mobilis
MKAAVITKDHTIEVKDTKLRPLKYGEALLEMEYCGVCHTDLHVKNGDFGDETGRITGHEGIGIVKQVGEGVTSLKVGDRASVAWFFKGCGHCEYCVSGNETLCRNVENAGYTVDGAMAEECIVVADYSVKVPDGLDPAVASSITCAGVTTYKAVKVSQIQPGQWLAIYGLGGLGNLALQYAKNVFNAKVIAIDVNDEQLAFAKELGADMVINPKNEDAAKIIQEKVGGAHATVVTAVAKSAFNSAVEAIRAGGRVVAVGLPPEKMDLSIPRLVLDGIEVLGSLVGTREDLKEAFQFAAEGKVKPKVTKRKVEEINQIFDEMEHGKFTGRMVVDFTHH

SEQ ID NO: 17 - DNA, 2619 bp, Thermoanaerobacter thermocopriae
  source 1..2619: mol_type = genomic DNA
atgcctactttattacaagaaaaaaaggaagcaaaagaaaaaacagaagtaaaagaaacaacagatgttaaaaaacaaatagacctattagtagaaagggcgaaaagagcccaagaaaaattcatgtcatacactcagcagcaaattgatgaaatagtcaaagctatggcactaacgggcatagaaaagcatgtagaactggcaagattagctcatgaagaaacaaaaatgggtgtttatgaagacaaaataacgaaaaatctctttgcagtagaatatgtgtacaattatataaaagacaaaaaaactgtaggcatcctcaaagaaaacttagaagaaaattatatggaagtggcagagcctgtaggaattatagccggagtaacacctgtcacaaaccctacttctacaacaatgttcaaatgcctaattgctattaaaacaagaaatccaataatttttagtttccatcccaaagcattaaaatgtagtatagaagcagcaaagaccatgtacgaggcagcattaaaggcgggtgctcccgaaggatgcataggttggattgaaacaccttcaattgaagcaacgcaacttctcatgacacatcccggtgtctcccttatcctcgcaacaggcggtgcaggaatggtaaaagctgcttatagctcaggaaaacccgcccttggcgtaggtcctggcaatgtcccctgctacattgaaaaaactgcaaatattaaaagagcggtctcagacctaatacttagcaaaacttttgacaatggcacagtatgcgcatcagaacaagctgtgataatagatgaagaaatagccaatgaagtaaaaaaattaatgagagaatatggttgctatttcttaaataaagaagaaactaaaaagttagaagaattcgctatagacaaaaacaccggtttaatgaatccagcagttgtgggtcagcctgcagtgaaaattgctcaaatggctggatttaaagttcctgaaaataccaaaatacttgtagctgaatatccagctgtaggtcctgaatatcctctatccagagaaaaactaagcccaatacttgctttatacacagtcaaagattacaaagaaggtataaaaagatgcgaagaaatgatacaattcggcggacttggtcactctgcggtaatacattctgaaaaccaacaaattattaatgaatttgcaaatagagtacaagcaagtagaatccttgtaaacgcccctgcttcacaaggcgctattggaaacatttataacacggctactccatctttgactttgggttgcggtacaatgggtggaaattcaacaacagataatgtaagtgtttataaccttataaatataaaacgagtttttataagaaaagagagaatgaaatggttcagagttccaccacaaatctattttgaaagagggtcaatacagtatctatcacaagtaaaaggcaaaaaagcctttattgtaacagaccctgcgatggttaaattaggttttgtagataaagtgacatatcaattagataaagcaaatattaaatatgaaattttctctgaagtagaaccagacccatcagttgacactgtagaaaaagggataaaaataatgaaggagttcgagcctgacttactaatagctataggtggtggttctgcaatagacgcagcaaagggaatgtggcttttttatgagtaccctgacacaaaatttgaagacttaaggttaaagttcatggacataagaaaaagaacttatagatttcctgaactcggcaaaaacgctttatttatcgcaataccaaccaccagcggtacaggttctgaagtcacagcctttgcagttataacagacaaaaagaaaaatataaagtaccctcttacagattacgaattgacaccagatattgctataatagaccctgactttgtcatgacaattccaccctctgtaactgcagatacaggtatggatgctttaactcatgccattgaagcttatgtatccgttatggcatcagactatacagacgccctcgcagaaaaagccataaaactgatatttgaatatctccctaaagcatataaaaacggacaagacaaagtcgcccgcgaaaagatgcacaatgcttcttgcatagcaggaatggcattcacaaatgcatttttaggaataaaccacagtatggcccacatacttggcgctaaattccaccttccccacggaagggcaaatgcgatacttctgccctatgtcatagaatacaatgctgagttacctaaaaaatttgcctcattcccacaatatgaatatcccaaagcagccgagaaatacgcagaaattgcaaaattcttaggacttcctgcatcaaccactgatgaaggagtaaaaagtctcattgaagcaataaaaaatctcatgaaagagttaaatcttcctcttacacttaaagatgcgggaataaacaaagaagaatttgaaaaacaaataatggaaatggctgatatagccttcaacgaccagtgcaccggttcaaatccaagaatgccattggtatcagaaattgcagaaatatatagaaaagcctatggagaataa

SEQ ID NO: 18 - protein, 872 aa, Thermoanaerobacter thermocopriae
MPTLLQEKKEAKEKTEVKETTDVKKQIDLLVERAKRAQEKFMSYTQQQIDEIVKAMALTGIEKHVELARLAHEETKMGVYEDKITKNLFAVEYVYNYIKDKKTVGILKENLEENYMEVAEPVGIIAGVTPVTNPTSTTMFKCLIAIKTRNPIIFSFHPKALKCSIEAAKTMYEAALKAGAPEGCIGWIETPSIEATQLLMTHPGVSLILATGGAGMVKAAYSSGKPALGVGPGNVPCYIEKTANIKRAVSDLILSKTFDNGTVCASEQAVIIDEEIANEVKKLMREYGCYFLNKEETKKLEEFAIDKNTGLMNPAVVGQPAVKIAQMAGFKVPENTKILVAEYPAVGPEYPLSREKLSPILALYTVKDYKEGIKRCEEMIQFGGLGHSAVIHSENQQIINEFANRVQASRILVNAPASQGAIGNIYNTATPSLTLGCGTMGGNSTTDNVSVYNLINIKRVFIRKERMKWFRVPPQIYFERGSIQYLSQVKGKKAFIVTDPAMVKLGFVDKVTYQLDKANIKYEIFSEVEPDPSVDTVEKGIKIMKEFEPDLLIAIGGGSAIDAAKGMWLFYEYPDTKFEDLRLKFMDIRKRTYRFPELGKNALFIAIPTTSGTGSEVTAFAVITDKKKNIKYPLTDYELTPDIAIIDPDFVMTIPPSVTADTGMDALTHAIEAYVSVMASDYTDALAEKAIKLIFEYLPKAYKNGQDKVAREKMHNASCIAGMAFTNAFLGINHSMAHILGAKFHLPHGRANAILLPYVIEYNAELPKKFASFPQYEYPKAAEKYAEIAKFLGLPASTTDEGVKSLIEAIKNLMKELNLPLTLKDAGINKEEFEKQIMEMADIAFNDQCTGSNPRMPLVSEIAEIYRKAYGE

SEQ ID NO: 19 - DNA, 2607 bp, Geobacillus stearothermophilus
  source 1..2607: mol_type = genomic DNA
atggctgttgatgaaaaagtattagaccaaaagaaagaagttacaaaaatgatcgatacgctcgtcgcgaatgcgcaaaaagcgttaaaagcgtttcgtgattacgatcaagaagcgattgatcatatcgtcaagcaaatggcgttagctggacttgacaaacatatgtatttagcgaagttagcgattgaagaaacaaaacgtggcgtgtatgaagataaaatcattaaaaacatttttgcgacagaatacatttatcataacatcaaatatgataaaaccgtcggcgttattcgcgaaaatgaacaagaaggtattattgaaattgctgagcctgttggagtcatcgctggggttacaccagtaacaaacccaacatcaactacgatgtttaaagcgcttatttcaatcaagacgcgcaatccaatcatttttgcgttccatccgtccgcgcaaaaatgcagcagtgaagcggcacgcattttacgtgatgcagcgattgcggccggtgcgccagaacattgtattcaatggatcgaaacaccttccgttgaagcaacgcaacaacttatgcatcaccctggtgtttcgcttattcttgcgacaggtggagcaggcatggtcaaagcagcatatagctcaggaaaaccagcattaggggttggacctggtaacgtaccttgttatattgaaaaaacagcaaatattaaacgcgcggtgaacgaccttattctttcaaaaacgtttgataacggaatgatttgtgcatctgaacaagcggtcattattgataaagaaatatatgatgcggtgaaaaacgaaatgatcgcaaacaaatgttactttttaaatgaagaagaaaagaaaaaagtcgaaaagcttgtcattaatgaaaatacgtgtgcagtaaacccgaatatcgtcggtaaaccagcatatgaaattgcaaaaatggccggtgtggacgttccagttgatacgaaaattcttgtcgcagaattaaaaagcgtcggtccgcaagagccgctttctcgtgaaaaattaagtcctgtattggcgtgctataaggtgaatagcacagaagaagggttaaaacgagcagaagaaatgcttgaatttggtggacttggccactccgctgtcattcattcggaaaatcaagacgtcattcttgaattcggtaagcgaatgaaagcaggacgaatcatctctaatgcaccatcttcacaaggagcgatcggggacatttacaacgcatacattccgtcattgacgctcggttgcggtacgtttggaggcaactccgtttcgacaaacgtgggtgcgacacacttaattaatattaaaaaattagcgagaaggaatgtaaacatgcaatggtttaaagttccaccaaaaatttattttgaaaaacatgcgacacaatatttagcgaaaatgccaaacatctcacgtgcctttatcgttacagacccaggtatggtgaagctcggctatgtcgataaagtgttatactatttgcgtaaacgtccagattatgtgcattgcgaaattttctcagaagttgaaccagatccatcaattgaaacagtgatgaaaggtgccgacatgatgcatgcgttccagccagacgtcatcatcgcgctcggcggtggttcggcgatggacgcggcgaaagcgatgtggctgttctatgaacatccaaataccgactttaatggcttaaaacaaaagtttttagatattcgtaaacgcgtatttaaatatccaaaactcggtcaaaaagcgcaatttgtcgcgattccaacaacatctggtacaggttcagaagtgacatcgtttgcggtcattacagataagaaaaataacgtcaaatatccgcttgctgactacgagttaacaccagatgtcgccatcgttgacccacaattcgtcatgacgatgccaaaacatattacagcggatacaggtatggacgtattaacacatgcgattgaagcgtacgtatcgaacatggcaaacgactacacagacggattagcactaaaagccattcaactcgtctttgaatatttgccacgcgcatacaaaaacggcaacgatgaagtggcgcgcgaaaaaatgcataacgcatcaacgattgccggtatggcattcgcgaacgcatttttaggcattaaccatagtttagcgcataaacttggcgcagaattccatattccgcacggacgtgcgaacacgattttaatgccgcacgtcattcgttataacgcgacaaaaccgaagaaatttgtagcgttccctaaatatgaacattttatcgcggataaacgctatgcggaaatcgcacgcattttaggattgccagcacgcacaacggaagaaggagtcgaaagcctcattcaagcgattatcaagcttgcaaaagagcttgaaatgccattaagcatcgcggaaacaggcgtcagcaaagaagagtttgaaagcaaagtcgaacaacttgctgaactagcttttgaagatcaatgtacaacagccaacccaaaattaccattagtcagcgaccttgccgacatttatcgccaagcgtataaaggggttgaatga

SEQ ID NO: 20 - protein, 868 aa, Geobacillus stearothermophilus
MAVDEKVLDQKKEVTKMIDTLVANAQKALKAFRDYDQEAIDHIVKQMALAGLDKHMYLAKLAIEETKRGVYEDKIIKNIFATEYIYHNIKYDKTVGVIRENEQEGIIEIAEPVGVIAGVTPVTNPTSTTMFKALISIKTRNPIIFAFHPSAQKCSSEAARILRDAAIAAGAPEHCIQWIETPSVEATQQLMHHPGVSLILATGGAGMVKAAYSSGKPALGVGPGNVPCYIEKTANIKRAVNDLILSKTFDNGMICASEQAVIIDKEIYDAVKNEMIANKCYFLNEEEKKKVEKLVINENTCAVNPNIVGKPAYEIAKMAGVDVPVDTKILVAELKSVGPQEPLSREKLSPVLACYKVNSTEEGLKRAEEMLEFGGLGHSAVIHSENQDVILEFGKRMKAGRIISNAPSSQGAIGDIYNAYIPSLTLGCGTFGGNSVSTNVGATHLINIKKLARRNVNMQWFKVPPKIYFEKHATQYLAKMPNISRAFIVTDPGMVKLGYVDKVLYYLRKRPDYVHCEIFSEVEPDPSIETVMKGADMMHAFQPDVIIALGGGSAMDAAKAMWLFYEHPNTDFNGLKQKFLDIRKRVFKYPKLGQKAQFVAIPTTSGTGSEVTSFAVITDKKNNVKYPLADYELTPDVAIVDPQFVMTMPKHITADTGMDVLTHAIEAYVSNMANDYTDGLALKAIQLVFEYLPRAYKNGNDEVAREKMHNASTIAGMAFANAFLGINHSLAHKLGAEFHIPHGRANTILMPHVIRYNATKPKKFVAFPKYEHFIADKRYAEIARILGLPARTTEEGVESLIQAIIKLAKELEMPLSIAETGVSKEEFESKVEQLAELAFEDQCTTANPKLPLVSDLADIYRQAYKGVE

SEQ ID NO: 21 - DNA, 35 bp, synthetic construct
  source 1..35: mol_type = other DNA
ttttataacccgggccatcgactgcacggtgcacc

SEQ ID NO: 22 - DNA, 35 bp, synthetic construct
  source 1..35: mol_type = other DNA
tgctagcactgtttcctgtgtgaaattgttatccg

SEQ ID NO: 23 - DNA, 38 bp, synthetic construct
  source 1..38: mol_type = other DNA
ggaaacagtgctagcagatctggaggagaaacgcatat

SEQ ID NO: 24 - DNA, 72 bp, synthetic construct
  source 1..72: mol_type = other DNA
cagtgcggccgcaagcttgtcgacggagctcgaattcggatccgatatcagcatatgcgtttctcctccaga

SEQ ID NO: 25 - DNA, 80 bp, synthetic construct
  source 1..80: mol_type = other DNA
acaagcttgcggccgcactgcagcaccatcaccaccatcattgataagatccggctgctaacaaagcccgaaaggaagct

SEQ ID NO: 26 - DNA, 63 bp, synthetic construct
  source 1..63: mol_type = other DNA
tatttgaatcgagttattgctcagcggtggcagcagccaactcagcttcctttcgggctttgt

SEQ ID NO: 27 - DNA, 35 bp, synthetic construct
  source 1..35: mol_type = other DNA
taactcgattcaaataaaacgaaaggctcagtcga

SEQ ID NO: 28 - DNA, 35 bp, synthetic construct
  source 1..35: mol_type = other DNA
cctagatccgcggagtttgtagaaacgcaaaaagg

SEQ ID NO: 29 - DNA, 35 bp, synthetic construct
  source 1..35: mol_type = other DNA
acaaactccgcggatctaggtgaagatcctttttg

SEQ ID NO: 30 - DNA, 35 bp, synthetic construct
  source 1..35: mol_type = other DNA
cgtccgcggccagcaaaaggccaggaaccgtaaaa

SEQ ID NO: 31 - DNA, 35 bp, synthetic construct
  source 1..35: mol_type = other DNA
ttgctggccgcggacgtagaaagcctgtccgcaga

SEQ ID NO: 32 - DNA, 35 bp, synthetic construct
  source 1..35: mol_type = other DNA
ggcccgggttataaaagccagtcattaggcctatc

SEQ ID NO: 33 - DNA, 35 bp, synthetic construct
  source 1..35: mol_type = other DNA
aattgtcagataggcctaatgactggcttttataa

SEQ ID NO: 34 - DNA, 35 bp, synthetic construct
  source 1..35: mol_type = other DNA
tgacgccagaagcattggtgcaccgtgcagtcgat

SEQ ID NO: 35 - DNA, 19 bp, synthetic construct
  source 1..19: mol_type = other DNA
gatctggaggagaaacgca

SEQ ID NO: 36 - DNA, 17 bp, synthetic construct
  source 1..17: mol_type = other DNA
tatgcgtttctcctcca

SEQ ID NO: 37 - DNA, 35 bp, synthetic construct
  source 1..35: mol_type = other DNA
gaggccatctaggccatgagtaagtctgacggaac

SEQ ID NO: 38 - DNA, 35 bp, synthetic construct
  source 1..35: mol_type = other DNA
atccggcacccatatctgaaccggacgcaaacccg

SEQ ID NO: 39 - DNA, 35 bp, synthetic construct
  source 1..35: mol_type = other DNA
ttcagatatgggtgccggatacccgccgcccgggc

SEQ ID NO: 40 - DNA, 35 bp, synthetic construct
  source 1..35: mol_type = other DNA
aaggccttcatggccttatttcgcgattcccaaga

SEQ ID NO: 41 - DNA, 36 bp, synthetic construct
  source 1..36: mol_type = other DNA
atgaaagtaacaaatgcatgcctactttattacaag

SEQ ID NO: 42 - DNA, 39 bp, synthetic construct
  source 1..39: mol_type = other DNA
gtcgacggagctcgaattcttattctccataggcttttc

SEQ ID NO: 43 - DNA, 44 bp, synthetic construct
  source 1..44: mol_type = other DNA
atctggaggagaaacgcatatgaaagtaacaaatgcagaagaac

SEQ ID NO: 44 - DNA, 44 bp, synthetic construct
  source 1..44: mol_type = other DNA
gtcgacggagctcgaattcttatttattattttcttcagtttcc

SEQ ID NO: 45 - DNA, 44 bp, synthetic construct
  source 1..44: mol_type = other DNA
atctggaggagaaacgcatatggaaaacaaagaaagaaagattg

SEQ ID NO: 46 - DNA, 44 bp, synthetic construct
  source 1..44: mol_type = other DNA
gtcgacggagctcgaattctcatgctctcttcgctccgactctg

SEQ ID NO: 47 - DNA, 43 bp, synthetic construct
  source 1..43: mol_type = other DNA
atgaaagtaacaaatgcatgcctaacttattacaagaaagaag

SEQ ID NO: 48 - DNA, 39 bp, synthetic construct; identical to SEQ ID NO: 42
  source 1..39: mol_type = other DNA

SEQ ID NO: 49 - DNA, 45 bp, synthetic construct
  source 1..45: mol_type = other DNA
atctggaggagaaacgcatatggcaatcgatgaaaaagttgttgg

SEQ ID NO: 50 - DNA, 40 bp, synthetic construct
  source 1..40: mol_type = other DNA
gtcgacggagctcgaattcttattttgcttcaacgccttc

SEQ ID NO: 51 - DNA, 43 bp, synthetic construct
  source 1..43: mol_type = other DNA
atctggaggagaaacgcatatgtccgaaagggttaaggtagcc

SEQ ID NO: 52 - DNA, 43 bp, synthetic construct
  source 1..43: mol_type = other DNA
gtcgacggagctcgaattctcacgccaccacctcctccacggg

SEQ ID NO: 53 - DNA, 44 bp, synthetic construct
  source 1..44: mol_type = other DNA
atctggaggagaaacgcatatgagagcagcagtcgtcagttctg

SEQ ID NO: 54 - DNA, 44 bp, synthetic construct
  source 1..44: mol_type = other DNA
gtcgacggagctcgaattcttatttcaacgacatatccaggacc

SEQ ID NO: 55 - DNA, 40 bp, synthetic construct
  source 1..40: mol_type = other DNA
gatctggaggagaaacgcatatgaaagcagccgtcataac

SEQ ID NO: 56 - DNA, 40 bp, synthetic construct
  source 1..40: mol_type = other DNA
tgtcgacggagctcgaattcctagtgatgggtaaaatcaa

SEQ ID NO: 57 - DNA, 45 bp, synthetic construct
  source 1..45: mol_type = other DNA
atgaaagtaacaaatgcatgcctaccttattacaagaaaaaaagg

SEQ ID NO: 58 - DNA, 43 bp, synthetic construct
  source 1..43: mol_type = other DNA
gtcgacggagctcgaattcctatatcagaatttccattatttg

SEQ ID NO: 59 - DNA, 47 bp, synthetic construct
  source 1..47: mol_type = other DNA
atctggaggagaaacgcatatggctgttgatgaaaaagtattagacc

SEQ ID NO: 60 - DNA, 46 bp, synthetic construct
  source 1..46: mol_type = other DNA
gtcgacggagctcgaattctcattcaacccctttatacgcttggcg

SEQ ID NO: 61 - DNA, 20 bp, synthetic construct
  source 1..20: mol_type = other DNA
gaattcgagctccgtcgaca

SEQ ID NO: 62 - DNA, 20 bp, synthetic construct
  source 1..20: mol_type = other DNA
atgcgtttctcctccagatc